European Patent Application EP 4 209 599 A1, published July 12, 2023. Title: Method of screening for active anticancer immune cytokines and Composition for preventing or treating cancer disease comprising IL-15 thereof. Applicant: Daegu Gyeongbuk Institute of Science and Technology Kyungpook National University. The sequence listing filed with the application follows.

SEQUENCE LISTING (24 sequences)

SEQ ID NO: 1 - DNA, 20 bp, Artificial Sequence
  H-Rab27a-f
aaaaggagaaaggggcatgt

SEQ ID NO: 2 - DNA, 20 bp, Artificial Sequence
  H-Rab27a-r
taatggggatggtgagaagc

SEQ ID NO: 3 - DNA, 20 bp, Artificial Sequence
  H-PD-L1-f
ggtcatcccagaactacctc

SEQ ID NO: 4 - DNA, 20 bp, Artificial Sequence
  H-PD-L1-r
agtgctacaccaaggcataa

SEQ ID NO: 5 - DNA, 20 bp, Artificial Sequence
  H-GAPDH-f
gaatttggctacagcaacag

SEQ ID NO: 6 - DNA, 20 bp, Artificial Sequence
  H-GAPDH-r
tgagggtctctctcttcctc

SEQ ID NO: 7 - DNA, 20 bp, Artificial Sequence
  H-Rab5-f
gcatgggtccctctcactaa

SEQ ID NO: 8 - DNA, 20 bp, Artificial Sequence
  H-Rab5-r
gtggagaaatgggctggtta

SEQ ID NO: 9 - DNA, 20 bp, Artificial Sequence
  H-Rab7-f
ccctgtttggattgcagagt

SEQ ID NO: 10 - DNA, 20 bp, Artificial Sequence
  H-Rab7-r
tgcaaatcaacgttttggaa

SEQ ID NO: 11 - DNA, 20 bp, Artificial Sequence
  M-Rab27a-f
ttcctgcttctgttcgacct

SEQ ID NO: 12 - DNA, 20 bp, Artificial Sequence
  M-Rab27a-r
tttcactgccctctggtctt

SEQ ID NO: 13 - DNA, 20 bp, Artificial Sequence
  M-PD-L1-f
agttcccaaaacatgaggat

SEQ ID NO: 14 - DNA, 20 bp, Artificial Sequence
  M-PD-L1-r
cacgtacaagtcctttggag

SEQ ID NO: 15 - DNA, 19 bp, Artificial Sequence
  M-GAPDH-f
tcaccaccatggagaaggc

SEQ ID NO: 16 - DNA, 20 bp, Artificial Sequence
  M-GAPDH-r
gctaagcagttggtggtgca

SEQ ID NO: 17 - DNA, 20 bp, Artificial Sequence
  M-Rab5-f
tctgctgttggcaaatcaag

SEQ ID NO: 18 - DNA, 20 bp, Artificial Sequence
  M-Rab5-r
tctcgcaaaggattcctcat

SEQ ID NO: 19 - DNA, 20 bp, Artificial Sequence
  M-Rab7-f
ggccttctacagaggtgcag

SEQ ID NO: 20 - DNA, 20 bp, Artificial Sequence
  M-Rab7-r
tctttgtggccacttgtctg

SEQ ID NO: 21 - DNA, 20 bp, Artificial Sequence
  M-PD-1-f
agaatcctggagacctcaac

SEQ ID NO: 22 - DNA, 20 bp, Artificial Sequence
  M-PD-1-r
atacccactagggcactcat

SEQ ID NO: 23 - DNA, 20 bp, Artificial Sequence
  M-CTLL-4-f
ggactccggaggtacaaagc

SEQ ID NO: 24 - DNA, 21 bp, Artificial Sequence
  M-CTLL-4-r
ttgggtcacctgtatggcttc